European Patent Specification EP 3 712 275 B1, published March 19, 2025. Title: METHOD OF DETECTING TARGET MOLECULE. Applicant: TOPPAN PRINTING CO., LTD. The sequence listing filed with the application follows.

SEQUENCE LISTING (6 sequences)

SEQ ID NO: 1 - DNA, 140 bp, Escherichia coli
acgttaaacaaaaaatcgtttcttatttggattgggataaataatatggctgtttattttgtaactggcaaattaggctctggaaagacgctcgttagcgttggtaagattcaggataaaattgtagctgggtgcaaaat

SEQ ID NO: 2 - DNA, 28 bp, Artificial Sequence
  Synthesized DNA named allele probe 1
cgcgccgagggcctaatttgccagttac

SEQ ID NO: 3 - DNA, 22 bp, Artificial Sequence
  Synthesized DNA named invader oligo 1
gctaacgagcgtctttccagat

SEQ ID NO: 4 - DNA, 34 bp, Artificial Sequence
  Synthesized oligonucleotide
  misc_feature (1)..(1): Labeled with Alexa488
  misc_feature (4)..(4): Labeled with Black hole quencher-1
ttctagccggttttccggctgagacctcggcgcg

SEQ ID NO: 5 - DNA, 24 bp, Artificial Sequence
  Synthesized DNA named allele probe 2
cgcgccgaggcgcagctcatgccc

SEQ ID NO: 6 - DNA, 18 bp, Artificial Sequence
  Synthesized DNA named invader oligo 2
ccaccgtgcactcatcaa